European Patent Application EP 4 177 269 A1, published May 10, 2023. Title: Method for Producing Antibody. Applicant: SYSMEX CORPORATION. Application EP. The sequence listing filed with the application follows.

SEQUENCE LISTING (18 sequences)

SEQ ID NO: 1 - protein, 451 aa, synthetic construct
  REGION 1..451: note = chimeric antibody
QVQLQQPGAELVKPGASVKMSCKASGYTFTSYNMHWVKQTPGRGLEWIGAIYPGNGDTSYNQKFKGKATLTADKSSSTAYMQLSSLTSEDSAVYYCARSTYYGGDWYFNVWGAGTTVTVSAASTKGPSVFPLAPSSKSTSGGTAALGCLVKDYFPEPVTVSWNSGALTSGVHTFPAVLQSSGLYSLSSVVTVPSSSLGTQTYICNVNHKPSNTKVDKKAEPKSCDKTHTCPPCPAPELLGGPSVFLFPPKPKDTLMISRTPEVTCVVVDVSHEDPEVKFNWYVDGVEVHNAKTKPREEQYNSTYRVVSVLTVLHQDWLNGKEYKCKVSNKALPAPIEKTISKAKGQPREPQVYTLPPSRDELTKNQVSLTCLVKGFYPSDIAVEWESNGQPENNYKTTPPVLDSDGSFFLYSKLTVDKSRWQQGNVFSCSVMHEALHNHYTQKSLSLSPGK

SEQ ID NO: 2 - protein, 213 aa, synthetic construct
  REGION 1..213: note = chimeric antibody
QIVLSQSPAILSASPGEKVTMTCRASSSVSYIHWFQQKPGSSPKPWIYATSNLASGVPVRFSGSGSGTSYSLTISRVEAEDAATYYCQQWTSNPPTFGGGTKLEIKRTVAAPSVFIFPPSDEQLKSGTASVVCLLNNFYPREAKVQWKVDNALQSGNSQESVTEQDSKDSTYSLSSTLTLSKADYEKHKVYACEVTHQGLSSPVTKSFNRGEC

SEQ ID NO: 3 - protein, 213 aa, synthetic construct
  REGION 1..213: note = modified antibody
QIVLSQSPAILSASPGEKVTMTCRASSSVSYIHWFQQKPGSSPKPWIYATSNLASGVPVRFRGRGRGTSYSLTISRVEAEDAATYYCQQWTSNPPTFGGGTKLEIKRTVAAPSVFIFPPSDEQLKSGTASVVCLLNNFYPREAKVQWKVDNALQSGNSQESVTEQDSKDSTYSLSSTLTLSKADYEKHKVYACEVTHQGLSSPVTKSFNRGEC

SEQ ID NO: 4 - protein, 213 aa, synthetic construct
  REGION 1..213: note = modified antibody
QIVLSQSPAILSASPGEKVTMTCRASSSVSYIHWFQQKPGSSPKPWIYATSNLASGVPVRFRGRGRGTRYRLTISRVEAEDAATYYCQQWTSNPPTFGGGTKLEIKRTVAAPSVFIFPPSDEQLKSGTASVVCLLNNFYPREAKVQWKVDNALQSGNSQESVTEQDSKDSTYSLSSTLTLSKADYEKHKVYACEVTHQGLSSPVTKSFNRGEC

SEQ ID NO: 5 - protein, 450 aa, synthetic construct
  REGION 1..450: note = humanized antibody
EVQLVESGGGLVQPGGSLRLSCAASGFNIKDTYIHWVRQAPGKGLEWVARIYPTNGYTRYADSVKGRFTISADTSKNTAYLQMNSLRAEDTAVYYCSRWGGDGFYAMDYWGQGTLVTVSSASTKGPSVFPLAPSSKSTSGGTAALGCLVKDYFPEPVTVSWNSGALTSGVHTFPAVLQSSGLYSLSSVVTVPSSSLGTQTYICNVNHKPSNTKVDKKVEPKSCDKTHTCPPCPAPELLGGPSVFLFPPKPKDTLMISRTPEVTCVVVDVSHEDPEVKFNWYVDGVEVHNAKTKPREEQYNSTYRVVSVLTVLHQDWLNGKEYKCKVSNKALPAPIEKTISKAKGQPREPQVYTLPPSRDELTKNQVSLTCLVKGFYPSDIAVEWESNGQPENNYKTTPPVLDSDGSFFLYSKLTVDKSRWQQGNVFSCSVMHEALHNHYTQKSLSLSPGK

SEQ ID NO: 6 - protein, 214 aa, synthetic construct
  REGION 1..214: note = humanized antibody
DIQMTQSPSSLSASVGDRVTITCRASQDVNTAVAWYQQKPGKAPKLLIYSASFLYSGVPSRFSGSRSGTDFTLTISSLQPEDFATYYCQQHYTTPPTFGQGTKVEIKRTVAAPSVFIFPPSDEQLKSGTASVVCLLNNFYPREAKVQWKVDNALQSGNSQESVTEQDSKDSTYSLSSTLTLSKADYEKHKVYACEVTHQGLSLPVTKSFNRGEC

SEQ ID NO: 7 - protein, 214 aa, synthetic construct
  REGION 1..214: note = modified antibody
DIQMTQSPSSLSASVGDRVTITCRASQDVNTAVAWYQQKPGKAPKLLIYSASFLYSGVPSRFSGRRRGTRFTLTISSLQPEDFATYYCQQHYTTPPTFGQGTKVEIKRTVAAPSVFIFPPSDEQLKSGTASVVCLLNNFYPREAKVQWKVDNALQSGNSQESVTEQDSKDSTYSLSSTLTLSKADYEKHKVYACEVTHQGLSLPVTKSFNRGEC

SEQ ID NO: 8 - protein, 214 aa, synthetic construct
  REGION 1..214: note = modified antibody
DIQMTQSPSSLSASVGDRVTITCRASQDVNTAVAWYQQKPGKAPKLLIYSASFLYSGVPSRFRGRRRGTRFTLTISSLQPEDFATYYCQQHYTTPPTFGQGTKVEIKRTVAAPSVFIFPPSDEQLKSGTASVVCLLNNFYPREAKVQWKVDNALQSGNSQESVTEQDSKDSTYSLSSTLTLSKADYEKHKVYACEVTHQGLSLPVTKSFNRGEC

SEQ ID NO: 9 - protein, 437 aa, Mus musculus
DVQLQESGPSLVKPSQTLSLTCSVTGDSITSDYWSWIRKFPGNRLEYMGYVSYSGSTYYNPSLKSRISITRDTSKNQYYLDLNSVTTEDTATYYCANWDGDYWGQGTLVTVSAAKTTPPSVYPLAPGSAAQTNSMVTLGCLVKGYFPEPVTVTWNSGSLSSGVHTFPAVLQSDLYTLSSSVTVPSSTWPSETVTCNVAHPASSTKVDKKIVPRDCGCKPCICTVPEVSSVFIFPPKPKDVLTITLTPKVTCVVVDISKDDPEVQFSWFVDDVEVHTAQTQPREEQFNSTFRSVSELPIMHQDWLNGKEFKCRVNSAAFPAPIEKTISKTKGRPKAPQVYTIPPPKEQMAKDKVSLTCMITDFFPEDITVEWQWNGQPAENYKNTQPIMDTDGSYFVYSKLNVQKSNWEAGNTFTCSVLHEGLHNHHTEKSLSHSPGK

SEQ ID NO: 10 - protein, 214 aa, Mus musculus [sequence omitted]

SEQ ID NO: 11 - protein, 214 aa, synthetic construct
  REGION 1..214: note = modified antibody
DIVLTQSPATLSVTPGNSVSLSCRASQSIGNNLHWYQQKSHESPRLLIKYASQSISGIPSRFRGRGRGTRFRLSINSVETEDFGMYFCQQSNSWPYTFGGGTKLEIKRADAAPTVSIFPPSSEQLTSGGASVVCFLNNFYPKDINVKWKIDGSERQNGVLNSWTDQDSKDSTYSMSSTLTLTKDEYERHNSYTCEATHKTSTSPIVKSFNRNEC

SEQ ID NO: 12 - protein, 449 aa, synthetic construct
  REGION 1..449: note = chimeric antibody
EVQLQQSGPELVKPGASVKMSCKASGYTFTSYVMHWVKQKPGQGLEWIGYINPYNDGTKYNEKFKGKATLTSDKSSSTAYMELSSLTSEDSAVYYCAREGYGNLERDCWGQGTSVTVSSASTKGPSVFPLAPSSKSTSGGTAALGCLVKDYFPEPVTVSWNSGALTSGVHTFPAVLQSSGLYSLSSVVTVPSSSLGTQTYICNVNHKPSNTKVDKKVEPKSCDKTHTCPPCPAPELLGGPSVFLFPPKPKDTLMISRTPEVTCVVVDVSHEDPEVKFNWYVDGVEVHNAKTKPREEQYNSTYRVVSVLTVLHQDWLNGKEYKCKVSNKALPAPIEKTISKAKGQPREPQVYTLPPSRDELTKNQVSLTCLVKGFYPSDIAVEWESNGQPENNYKTTPPVLDSDGSFFLYSKLTVDKSRWQQGNVFSCSVMHEALHNHYTQKSLSLSPGK

SEQ ID NO: 13 - protein, 218 aa, synthetic construct
  REGION 1..218: note = chimeric antibody
DIVLTQSPASLAVSLGQRATISCRASESVDGFGISFMNWFQQKPGQPPKLLIYVASNQGSGVPARFSGSGSGTDFSLNIHPMEEDDSAMYFCQQSKEVPWTFGGGTKLEIKRTVAAPSVFIFPPSDEQLKSGTASVVCLLNNFYPREAKVQWKVDNALQSGNSQESVTEQDSKDSTYSLSSTLTLSKADYEKHKVYACEVTHQGLSSPVTMSFNRGEC

SEQ ID NO: 14 - protein, 218 aa, synthetic construct
  REGION 1..218: note = modified antibody
DIVLTQSPASLAVSLGQRATISCRASESVDGFGISFMNWFQQKPGQPPKLLIYVASNQGSGVPARFRGRGRGTRFRLNIHPMEEDDSAMYFCQQSKEVPWTFGGGTKLEIKRTVAAPSVFIFPPSDEQLKSGTASVVCLLNNFYPREAKVQWKVDNALQSGNSQESVTEQDSKDSTYSLSSTLTLSKADYEKHKVYACEVTHQGLSSPVTMSFNRGEC

SEQ ID NO: 15 - protein, 450 aa, synthetic construct
  REGION 1..450: note = chimeric antibody
EVKLVESGGGLVKPGGSLKLSCAASGFTFNNYAMSWVRQTPEKRLEWVASISSGGNTYYPDSVKGRFTLSRDNARNILYLQMSRLRSEDTAMYYCARDKLRLPNWYFDVWGAGTTVTVSSASTKGPSVFPLAPSSKSTSGGTAALGCLVKDYFPEPVTVSWNSGALTSGVHTFPAVLQSSGLYSLSSVVTVPSSSLGTQTYICNVNHKPSNTKVDKKVEPKSCDKTHTCPPCPAPELLGGPSVFLFPPKPKDTLMISRTPEVTCVVVDVSHEDPEVKFNWYVDGVEVHNAKTKPREEQYNSTYRVVSVLTVLHQDWLNGKEYKCKVSNKALPAPIEKTISKAKGQPREPQVYTLPPSRDELTKNQVSLTCLVKGFYPSDIAVEWESNGQPENNYKTTPPVLDSDGSFFLYSKLTVDKSRWQQGNVFSCSVMHEALHNHYTQKSLSLSPGK

SEQ ID NO: 16 - protein, 218 aa, synthetic construct
  REGION 1..218: note = chimeric antibody
DIVLTQSPPSLAVSLGQRATISCKASQSVDYDGDSYMNWYQQKPGQPPKVLIYGASNLESGIPARFSGSGSGTDFTLNIYPVEEEDAATYYCQQSNEDPPTFGGGTKLEIKRTVAAPSVFIFPPSDEQLKSGTASVVCLLNNFYPREAKVQWKVDNALQSGNSQESVTEQDSKDSTYSLSSTLTLSKADYEKHKVYACEVTHQGLSSPVTMSFNRGEC

SEQ ID NO: 17 - protein, 218 aa, synthetic construct
  REGION 1..218: note = modified antibody
DIVLTQSPPSLAVSLGQRATISCKASQSVDYDGDSYMNWYQQKPGQPPKVLIYGASNLESGIPARFRGRGRGTDFTLNIYPVEEEDAATYYCQQSNEDPPTFGGGTKLEIKRTVAAPSVFIFPPSDEQLKSGTASVVCLLNNFYPREAKVQWKVDNALQSGNSQESVTEQDSKDSTYSLSSTLTLSKADYEKHKVYACEVTHQGLSSPVTMSFNRGEC

SEQ ID NO: 18 - protein, 218 aa, synthetic construct
  REGION 1..218: note = modified antibody
DIVLTQSPPSLAVSLGQRATISCKASQSVDYDGDSYMNWYQQKPGQPPKVLIYGASNLESGIPARFRGRGRGTRFTLNIYPVEEEDAATYYCQQSNEDPPTFGGGTKLEIKRTVAAPSVFIFPPSDEQLKSGTASVVCLLNNFYPREAKVQWKVDNALQSGNSQESVTEQDSKDSTYSLSSTLTLSKADYEKHKVYACEVTHQGLSSPVTMSFNRGEC